European Patent Specification EP 3 572 423 B1, published December 6, 2023. Title: ANTI-HUMAN PAPILLOMAVIRUS 16 E6 T CELL RECEPTORS. Applicant: THE UNITED STATES OF AMERICA, AS REPRESENTED BY THE SECRETARY, DEPARTMENT OF HEALTH AND HUMAN SERVICES. Application 14 748 353.1. The sequence listing filed with the application follows.

SEQUENCE LISTING (39 sequences)

SEQ ID NO: 1 - protein, 158 aa, Artificial Sequence
  Synthetic
MHQKRTAMFQDPQERPRKLPQLCTELQTTIHDIILECVYCKQQLLRREVYDFAFRDLCIVYRDGNPYAVCDKCLKFYSKISEYRHYCYSLYGTTLEQQYNKPLCDLLIRCINCQKPLCPEEKQRHLDKKQRFHNIRGRWTGRCMSCCRSSRTRRETQL

SEQ ID NO: 2 - protein, 10 aa, Artificial Sequence
  Synthetic
TIHDIILECV

SEQ ID NO: 3 - protein, 5 aa, Artificial Sequence
  Synthetic
SIFNT

SEQ ID NO: 4 - protein, 7 aa, Artificial Sequence
  Synthetic
LYKAGEL

SEQ ID NO: 5 - protein, 13 aa, Artificial Sequence
  Synthetic
AGHPSSNSGYALN

SEQ ID NO: 6 - protein, 5 aa, Artificial Sequence
  Synthetic
SGHVS

SEQ ID NO: 7 - protein, 6 aa, Artificial Sequence
  Synthetic
FNYEAQ

SEQ ID NO: 8 - protein, 14 aa, Artificial Sequence
  Synthetic
ASSSQTGARTDTQY

SEQ ID NO: 9 - protein, 131 aa, Artificial Sequence
  Synthetic
MLLEHLLIILWMQLTWVSGQQLNQSPQSMFIQEGEDVSMNCTSSSIFNTWLWYKQDPGEGPVLLIALYKAGELTSNGRLTAQFGITRKDSFLNISASIPSDVGIYFCAGHPSSNSGYALNFGKGTSLLVTP

SEQ ID NO: 10 - protein, 135 aa, Artificial Sequence
  Synthetic
MGTSLLCWVVLGFLGTDHTGAGVSQSPRYKVTKRGQDVALRCDPISGHVSLYWYRQALGQGPEFLTYFNYEAQQDKSGLPNDRFSAERPEGSISTLTIQRTEQRDSAMYRCASSSQTGARTDTQYFGPGTRLTVL

SEQ ID NO: 11 - protein, 272 aa, Artificial Sequence
  Synthetic
MLLEHLLIILWMQLTWVSGQQLNQSPQSMFIQEGEDVSMNCTSSSIFNTWLWYKQDPGEGPVLLIALYKAGELTSNGRLTAQFGITRKDSFLNISASIPSDVGIYFCAGHPSSNSGYALNFGKGTSLLVTPHIQNPDPAVYQLRDSKSSDKSVCLFTDFDSQTNVSQSKDSDVYITDKTVLDMRSMDFKSNSAVAWSNKSDFACANAFNNSIIPEDTFFPSPESSCDVKLVEKSFETDTNLNFQNLSVIGFRILLLKVAGFNLLMTLRLWSS

SEQ ID NO: 12 - protein, 314 aa, Artificial Sequence [sequence omitted]

SEQ ID NO: 13 - protein, 141 aa, Artificial Sequence
  Synthetic
HIQNPDPAVYQLRDSKSSDKSVCLFTDFDSQTNVSQSKDSDVYITDKTVLDMRSMDFKSNSAVAWSNKSDFACANAFNNSIIPEDTFFPSPESSCDVKLVEKSFETDTNLNFQNLSVIGFRILLLKVAGFNLLMTLRLWSS

SEQ ID NO: 14 - protein, 179 aa, Artificial Sequence
  Synthetic
EDLKNVFPPEVAVFEPSEAEISHTQKATLVCLATGFYPDHVELSWWVNGKEVHSGVSTDPQPLKEQPALNDSRYCLSSRLRVSATFWQNPRNHFRCQVQFYGLSENDEWTQDRAKPVTQIVSAEAWGRADCGFTSESYQQGVLSATILYEILLGKATLYAVLVSALVLMAMVKRKDSRG

SEQ ID NO: 15 - protein, 137 aa, Artificial Sequence
  Synthetic
DIQNPEPAVYQLKDPRSQDSTLCLFTDFDSQINVPKTMESGTFITDKTVLDMKAMDSKSNGAIAWSNQTSFTCQDIFKETNATYPSSDVPCDATLTEKSFETDMNLNFQNLSVMGLRILLLKVAGFNLLMTLRLWSS

SEQ ID NO: 16 - protein, 173 aa, Artificial Sequence
  Synthetic
EDLRNVTPPKVSLFEPSKAEIANKQKATLVCLARGFFPDHVELSWWVNGKEVHSGVSTDPQAYKESNYSYCLSSRLRVSATFWHNPRNHFRCQVQFHGLSEEDKWPEGSPKPVTQNISAEAWGRADCGITSASYQQGVLSATILYEILLGKATLYAVLVSTLVVMAMVKRKNS

SEQ ID NO: 17 - protein, 268 aa, Artificial Sequence
  Synthetic
MLLEHLLIILWMQLTWVSGQQLNQSPQSMFIQEGEDVSMNCTSSSIFNTWLWYKQDPGEGPVLLIALYKAGELTSNGRLTAQFGITRKDSFLNISASIPSDVGIYFCAGHPSSNSGYALNFGKGTSLLVTPDIQNPEPAVYQLKDPRSQDSTLCLFTDFDSQINVPKTMESGTFITDKTVLDMKAMDSKSNGAIAWSNQTSFTCQDIFKETNATYPSSDVPCDATLTEKSFETDMNLNFQNLSVMGLRILLLKVAGFNLLMTLRLWSS

SEQ ID NO: 18 - protein, 308 aa, Artificial Sequence
  Synthetic
MGTSLLCWVVLGFLGTDHTGAGVSQSPRYKVTKRGQDVALRCDPISGHVSLYWYRQALGQGPEFLTYFNYEAQQDKSGLPNDRFSAERPEGSISTLTIQRTEQRDSAMYRCASSSQTGARTDTQYFGPGTRLTVLEDLRNVTPPKVSLFEPSKAEIANKQKATLVCLARGFFPDHVELSWWVNGKEVHSGVSTDPQAYKESNYSYCLSSRLRVSATFWHNPRNHFRCQVQFHGLSEEDKWPEGSPKPVTQNISAEAWGRADCGITSASYQQGVLSATILYEILLGKATLYAVLVSTLVVMAMVKRKNS

SEQ ID NO: 19 - DNA, 393 bp, Artificial Sequence
  Synthetic
atgctccttgaacatttattaataatcttgtggatgcagctgacatgggtcagtggtcaacagctgaatcagagtcctcaatctatgtttatccaggaaggagaagatgtctccatgaactgcacttcttcaagcatatttaacacctggctatggtacaagcaggaccctggggaaggtcctgtcctcttgatagccttatataaggctggtgaattgacctcaaatggaagactgactgctcagtttggtataaccagaaaggacagcttcctgaatatctcagcatccatacctagtgatgtaggcatctacttctgtgctgggcacccttcctcaaattccgggtatgcactcaacttcggcaaaggcacctcgctgttggtcacaccc

SEQ ID NO: 20 - DNA, 405 bp, Artificial Sequence
  Synthetic
atgggcaccagtctcctatgctgggtggtcctgggtttcctagggacagatcacacaggtgctggagtctcccagtctcccaggtacaaagtcacaaagaggggacaggatgtagctctcaggtgtgatccaatttcgggtcatgtatccctttattggtaccgacaggccctggggcagggcccagagtttctgacttacttcaattatgaagcccaacaagacaaatcagggctgcccaatgatcggttctctgcagagaggcctgagggatccatctccactctgacgatccagcgcacagagcagcgggactcggccatgtatcgctgtgccagcagctcccagacaggggcccgcacagatacgcagtattttggcccaggcacccggctgacagtgctc

SEQ ID NO: 21 - DNA, 819 bp, Artificial Sequence
  Synthetic
atgctccttgaacatttattaataatcttgtggatgcagctgacatgggtcagtggtcaacagctgaatcagagtcctcaatctatgtttatccaggaaggagaagatgtctccatgaactgcacttcttcaagcatatttaacacctggctatggtacaagcaggaccctggggaaggtcctgtcctcttgatagccttatataaggctggtgaattgacctcaaatggaagactgactgctcagtttggtataaccagaaaggacagcttcctgaatatctcagcatccatacctagtgatgtaggcatctacttctgtgctgggcacccttcctcaaattccgggtatgcactcaacttcggcaaaggcacctcgctgttggtcacaccccatatccagaaccctgaccctgccgtgtaccagctgagagactctaaatccagtgacaagtctgtctgcctattcaccgattttgattctcaaacaaatgtgtcacaaagtaaggattctgatgtgtatatcacagacaaaactgtgctagacatgaggtctatggacttcaagagcaacagtgctgtggcctggagcaacaaatctgactttgcatgtgcaaacgccttcaacaacagcattattccagaagacaccttcttccccagcccagaaagttcctgtgatgtcaagctggtcgagaaaagctttgaaacagatacgaacctaaactttcaaaacctgtcagtgattgggttccgaatcctcctcctgaaagtggccgggtttaatctgctcatgacgctgcggctgtggtccagctga

SEQ ID NO: 22 - DNA, 945 bp, Artificial Sequence
  Synthetic
atgggcaccagtctcctatgctgggtggtcctgggtttcctagggacagatcacacaggtgctggagtctcccagtctcccaggtacaaagtcacaaagaggggacaggatgtagctctcaggtgtgatccaatttcgggtcatgtatccctttattggtaccgacaggccctggggcagggcccagagtttctgacttacttcaattatgaagcccaacaagacaaatcagggctgcccaatgatcggttctctgcagagaggcctgagggatccatctccactctgacgatccagcgcacagagcagcgggactcggccatgtatcgctgtgccagcagctcccagacaggggcccgcacagatacgcagtattttggcccaggcacccggctgacagtgctcgaggacctgaaaaacgtgttcccacccgaggtcgctgtgtttgagccatcagaagcagagatctcccacacccaaaaggccacactggtgtgcctggccacaggcttctaccccgaccacgtggagctgagctggtgggtgaatgggaaggaggtgcacagtggggtcagcacagacccgcagcccctcaaggagcagcccgccctcaatgactccagatactgcctgagcagccgcctgagggtctcggccaccttctggcagaacccccgcaaccacttccgctgtcaagtccagttctacgggctctcggagaatgacgagtggacccaggatagggccaaacctgtcacccagatcgtcagcgccgaggcctggggtagagcagactgtggcttcacctccgagtcttaccagcaaggggtcctgtctgccaccatcctctatgagatcttgctagggaaggccaccttgtatgccgtgctggtcagtgccctcgtgctgatggccatggtcaagagaaaggattccagaggctag

SEQ ID NO: 23 - DNA, 426 bp, Artificial Sequence
  Synthetic
catatccagaaccctgaccctgccgtgtaccagctgagagactctaaatccagtgacaagtctgtctgcctattcaccgattttgattctcaaacaaatgtgtcacaaagtaaggattctgatgtgtatatcacagacaaaactgtgctagacatgaggtctatggacttcaagagcaacagtgctgtggcctggagcaacaaatctgactttgcatgtgcaaacgccttcaacaacagcattattccagaagacaccttcttccccagcccagaaagttcctgtgatgtcaagctggtcgagaaaagctttgaaacagatacgaacctaaactttcaaaacctgtcagtgattgggttccgaatcctcctcctgaaagtggccgggtttaatctgctcatgacgctgcggctgtggtccagctga

SEQ ID NO: 24 - DNA, 540 bp, Artificial Sequence
  Synthetic
gaggacctgaaaaacgtgttcccacccgaggtcgctgtgtttgagccatcagaagcagagatctcccacacccaaaaggccacactggtgtgcctggccacaggcttctaccccgaccacgtggagctgagctggtgggtgaatgggaaggaggtgcacagtggggtcagcacagacccgcagcccctcaaggagcagcccgccctcaatgactccagatactgcctgagcagccgcctgagggtctcggccaccttctggcagaacccccgcaaccacttccgctgtcaagtccagttctacgggctctcggagaatgacgagtggacccaggatagggccaaacctgtcacccagatcgtcagcgccgaggcctggggtagagcagactgtggcttcacctccgagtcttaccagcaaggggtcctgtctgccaccatcctctatgagatcttgctagggaaggccaccttgtatgccgtgctggtcagtgccctcgtgctgatggccatggtcaagagaaaggattccagaggctag

SEQ ID NO: 25 - DNA, 414 bp, Artificial Sequence
  Synthetic
gacatccagaacccagaacctgctgtgtaccagttaaaagatcctcggtctcaggacagcaccctctgcctgttcaccgactttgactcccaaatcaatgtgccgaaaaccatggaatctggaacgttcatcactgacaaaactgtgctggacatgaaagctatggattccaagagcaatggggccattgcctggagcaaccagacaagcttcacctgccaagatatcttcaaagagaccaacgccacctaccccagttcagacgttccctgtgatgccacgttgactgagaaaagctttgaaacagatatgaacctaaactttcaaaacctgtcagttatgggactccgaatcctcctgctgaaagtagccggatttaacctgctcatgacgctgaggctgtggtccagttga

SEQ ID NO: 26 - DNA, 522 bp, Artificial Sequence
  Synthetic
gaggatctgagaaatgtgactccacccaaggtctccttgtttgagccatcaaaagcagagattgcaaacaaacaaaaggctaccctcgtgtgcttggccaggggcttcttccctgaccacgtggagctgagctggtgggtgaatggcaaggaggtccacagtggggtcagcacggaccctcaggcctacaaggagagcaattatagctactgcctgagcagccgcctgagggtctctgctaccttctggcacaatcctcgcaaccacttccgctgccaagtgcagttccatgggctttcagaggaggacaagtggccagagggctcacccaaacctgtcacacagaacatcagtgcagaggcctggggccgagcagactgtgggattacctcagcatcctatcaacaaggggtcttgtctgccaccatcctctatgagatcctgctagggaaagccaccctgtatgctgtgcttgtcagtacactggtggtgatggctatggtcaaaagaaagaattcatga

SEQ ID NO: 27 - DNA, 807 bp, Artificial Sequence
  Synthetic
atgctccttgaacatttattaataatcttgtggatgcagctgacatgggtcagtggtcaacagctgaatcagagtcctcaatctatgtttatccaggaaggagaagatgtctccatgaactgcacttcttcaagcatatttaacacctggctatggtacaagcaggaccctggggaaggtcctgtcctcttgatagccttatataaggctggtgaattgacctcaaatggaagactgactgctcagtttggtataaccagaaaggacagcttcctgaatatctcagcatccatacctagtgatgtaggcatctacttctgtgctgggcacccttcctcaaattccgggtatgcactcaacttcggcaaaggcacctcgctgttggtcacacccgacatccagaacccagaacctgctgtgtaccagttaaaagatcctcggtctcaggacagcaccctctgcctgttcaccgactttgactcccaaatcaatgtgccgaaaaccatggaatctggaacgttcatcactgacaaaactgtgctggacatgaaagctatggattccaagagcaatggggccattgcctggagcaaccagacaagcttcacctgccaagatatcttcaaagagaccaacgccacctaccccagttcagacgttccctgtgatgccacgttgactgagaaaagctttgaaacagatatgaacctaaactttcaaaacctgtcagttatgggactccgaatcctcctgctgaaagtagccggatttaacctgctcatgacgctgaggctgtggtccagttga

SEQ ID NO: 28 - DNA, 927 bp, Artificial Sequence
  Synthetic'
atgggcaccagtctcctatgctgggtggtcctgggtttcctagggacagatcacacaggtgctggagtctcccagtctcccaggtacaaagtcacaaagaggggacaggatgtagctctcaggtgtgatccaatttcgggtcatgtatccctttattggtaccgacaggccctggggcagggcccagagtttctgacttacttcaattatgaagcccaacaagacaaatcagggctgcccaatgatcggttctctgcagagaggcctgagggatccatctccactctgacgatccagcgcacagagcagcgggactcggccatgtatcgctgtgccagcagctcccagacaggggcccgcacagatacgcagtattttggcccaggcacccggctgacagtgctcgaggatctgagaaatgtgactccacccaaggtctccttgtttgagccatcaaaagcagagattgcaaacaaacaaaaggctaccctcgtgtgcttggccaggggcttcttccctgaccacgtggagctgagctggtgggtgaatggcaaggaggtccacagtggggtcagcacggaccctcaggcctacaaggagagcaattatagctactgcctgagcagccgcctgagggtctctgctaccttctggcacaatcctcgcaaccacttccgctgccaagtgcagttccatgggctttcagaggaggacaagtggccagagggctcacccaaacctgtcacacagaacatcagtgcagaggcctggggccgagcagactgtgggattacctcagcatcctatcaacaaggggtcttgtctgccaccatcctctatgagatcctgctagggaaagccaccctgtatgctgtgcttgtcagtacactggtggtgatggctatggtcaaaagaaagaattcatga

SEQ ID NO: 29 - DNA, 1815 bp, Artificial Sequence
  Synthetic
atggcccttgaacatctgttgataatactgtggatgcaacttacctgggtatctggtcagcaattgaaccagtctccacagtccatgtttatccaagaaggggaggacgtgtccatgaattgtacaagctccagtatcttcaacacgtggctgtggtacaaacaggatcctggggaaggaccagtactgttgatagccctctataaggcgggcgaactgacatccaatggaagactcacagcccaattcggaattacccggaaggattctttcctcaacatctccgcgagtattccatctgatgtaggaatatacttctgtgcagggcatccgtctagcaacagtggatatgccctcaattttggaaagggcacctccctgctggttaccccagacattcagaaccccgaaccagccgtatatcagttgaaggacccaagatctcaggatagtacactctgtttgtttacggactttgactcacaaatcaacgtcccgaagactatggaaagtggtacgttcatcacagataagacggttctggacatgaaggctatggactcaaagagcaacggggcaattgcttggtccaaccagacaagctttacctgtcaggacatttttaaggagactaatgctacttatccctccagcgacgttccgtgtgatgcgactcttaccgagaagtcttttgagaccgatatgaatctcaacttccagaatctgtcagtgatgggtctgcggatcctgcttctgaaggttgcaggattcaatcttcttatgactctccggctctggtcttcaagagccaaaagaagtggttctggcgcgacgaattttagtttgcttaagcaagccggagatgtggaggaaaatcctggaccgatgggcacaagtttgctgtgctgggttgtgttgggctttctgggtacagatcatactggggcgggagtctctcaaagcccccgatacaaagtcactaaaagagggcaggatgtcgcgcttcgctgtgatcccattagcgggcatgtctccctttattggtaccggcaggctttgggacaaggaccggagttcctcacttacttcaactacgaagcgcagcaggacaagtccggtctgcctaatgatagattcagcgccgagagaccggagggcagtatctctactcttacgatacaaagaacggagcagcgagactctgctatgtatagatgtgcaagttctagccagacgggtgctcgcacggacactcaatatttcggtcctggtacaagattgaccgtcttggaggatctccggaacgtcaccccaccaaaggtcagtttgtttgagccatcaaaggcggagatcgccaacaaacagaaagctacgctcgtgtgtttggctcggggcttcttcccagaccacgtagaactttcctggtgggtcaatggaaaggaggttcattccggagtgtccactgatccccaagcgtacaaggaatccaactatagctactgtctctcatctcggctccgggtgagtgcgacattctggcataatcctcggaaccactttcgatgccaagtgcagtttcatgggttgagcgaggaagacaagtggcccgagggcagtcctaaaccagtcactcaaaacataagcgccgaggcatggggtagagccgattgtgggattactagcgcttcataccaacaaggggtattgagcgctacaattctttacgaaattctcctcggcaaggcgacgctctacgccgtactggtgtctactctcgtggttatggcaatggtgaaacggaaaaacagctaatga

SEQ ID NO: 30 - DNA, 7325 bp, Artificial Sequence
  Synthetic
ccatggcccttgaacatctgttgataatactgtggatgcaacttacctgggtatctggtcagcaattgaaccagtctccacagtccatgtttatccaagaaggggaggacgtgtccatgaattgtacaagctccagtatcttcaacacgtggctgtggtacaaacaggatcctggggaaggaccagtactgttgatagccctctataaggcgggcgaactgacatccaatggaagactcacagcccaattcggaattacccggaaggattctttcctcaacatctccgcgagtattccatctgatgtaggaatatacttctgtgcagggcatccgtctagcaacagtggatatgccctcaattttggaaagggcacctccctgctggttaccccagacattcagaaccccgaaccagccgtatatcagttgaaggacccaagatctcaggatagtacactctgtttgtttacggactttgactcacaaatcaacgtcccgaagactatggaaagtggtacgttcatcacagataagacggttctggacatgaaggctatggactcaaagagcaacggggcaattgcttggtccaaccagacaagctttacctgtcaggacatttttaaggagactaatgctacttatccctccagcgacgttccgtgtgatgcgactcttaccgagaagtcttttgagaccgatatgaatctcaacttccagaatctgtcagtgatgggtctgcggatcctgcttctgaaggttgcaggattcaatcttcttatgactctccggctctggtcttcaagagccaaaagaagtggttctggcgcgacgaattttagtttgcttaagcaagccggagatgtggaggaaaatcctggaccgatgggcacaagtttgctgtgctgggttgtgttgggctttctgggtacagatcatactggggcgggagtctctcaaagcccccgatacaaagtcactaaaagagggcaggatgtcgcgcttcgctgtgatcccattagcgggcatgtctccctttattggtaccggcaggctttgggacaaggaccggagttcctcacttacttcaactacgaagcgcagcaggacaagtccggtctgcctaatgatagattcagcgccgagagaccggagggcagtatctctactcttacgatacaaagaacggagcagcgagactctgctatgtatagatgtgcaagttctagccagacgggtgctcgcacggacactcaatatttcggtcctggtacaagattgaccgtcttggaggatctccggaacgtcaccccaccaaaggtcagtttgtttgagccatcaaaggcggagatcgccaacaaacagaaagctacgctcgtgtgtttggctcggggcttcttcccagaccacgtagaactttcctggtgggtcaatggaaaggaggttcattccggagtgtccactgatccccaagcgtacaaggaatccaactatagctactgtctctcatctcggctccgggtgagtgcgacattctggcataatcctcggaaccactttcgatgccaagtgcagtttcatgggttgagcgaggaagacaagtggcccgagggcagtcctaaaccagtcactcaaaacataagcgccgaggcatggggtagagccgattgtgggattactagcgcttcataccaacaaggggtattgagcgctacaattctttacgaaattctcctcggcaaggcgacgctctacgccgtactggtgtctactctcgtggttatggcaatggtgaaacggaaaaacagctaatgagaattctgcagtcgacggtaccgcgggcccgggatccgataaaataaaagattttatttagtctccagaaaaaggggggaatgaaagaccccacctgtaggtttggcaagctagcttaagtaacgccattttgcaaggcatggaaaatacataactgagaatagagaagttcagatcaaggttaggaacagagagacagcagaatatgggccaaacaggatatctgtggtaagcagttcctgccccggctcagggccaagaacagatggtccccagatgcggtcccgccctcagcagtttctagagaaccatcagatgtttccagggtgccccaaggacctgaaaatgaccctgtgccttatttgaactaaccaatcagttcgcttctcgcttctgttcgcgcgcttctgctccccgagctcaataaaagagcccacaacccctcactcggcgcgccagtcctccgatagactgcgtcgcccgggtacccgtgtatccaataaaccctcttgcagttgcatccgacttgtggtctcgctgttccttgggagggtctcctctgagtgattgactacccgtcagcgggggtctttcatgggtaacagtttcttgaagttggagaacaacattctgagggtaggagtcgaatattaagtaatcctgactcaattagccactgttttgaatccacatactccaatactcctgaaatccatcgatggagttcattatggacagcgcagaaagagctggggagaattgtgaaattgttatccgctcacaattccacacaacatacgagccggaagcataaagtgtaaagcctggggtgcctaatgagtgagctaactcacattaattgcgttgcgctcactgcccgctttccagtcgggaaacctgtcgtgccagctgcattaatgaatcggccaacgcgcggggagaggcggtttgcgtattgggcgctcttccgcttcctcgctcactgactcgctgcgctcggtcgttcggctgcggcgagcggtatcagctcactcaaaggcggtaatacggttatccacagaatcaggggataacgcaggaaagaacatgtgagcaaaaggccagcaaaaggccaggaaccgtaaaaaggccgcgttgctggcgtttttccataggctccgcccccctgacgagcatcacaaaaatcgacgctcaagtcagaggtggcgaaacccgacaggactataaagataccaggcgtttccccctggaagctccctcgtgcgctctcctgttccgaccctgccgcttaccggatacctgtccgcctttctcccttcgggaagcgtggcgctttctcatagctcacgctgtaggtatctcagttcggtgtaggtcgttcgctccaagctgggctgtgtgcacgaaccccccgttcagcccgaccgctgcgccttatccggtaactatcgtcttgagtccaacccggtaagacacgacttatcgccactggcagcagccactggtaacaggattagcagagcgaggtatgtaggcggtgctacagagttcttgaagtggtggcctaactacggctacactagaagaacagtatttggtatctgcgctctgctgaagccagttaccttcggaaaaagagttggtagctcttgatccggcaaacaaaccaccgctggtagcggtggtttttttgtttgcaagcagcagattacgcgcagaaaaaaaggatctcaagaagatcctttgatcttttctacggggtctgacgctcagtggaacgaaaactcacgttaagggattttggtcatgagattatcaaaaaggatcttcacctagatccttttaaattaaaaatgaagttttaaatcaatctaaagtatatatgagtaaacttggtctgacagttaccaatgcttaatcagtgaggcacctatctcagcgatctgtctatttcgttcatccatagttgcctgactccccgtcgtgtagataactacgatacgggagggcttaccatctggccccagtgctgcaatgataccgcgagacccacgctcaccggctccagatttatcagcaataaaccagccagccggaagggccgagcgcagaagtggtcctgcaactttatccgcctccatccagtctattaattgttgccgggaagctagagtaagtagttcgccagttaatagtttgcgcaacgttgttgccattgctacaggcatcgtggtgtcacgctcgtcgtttggtatggcttcattcagctccggttcccaacgatcaaggcgagttacatgatcccccatgttgtgcaaaaaagcggttagctccttcggtcctccgatcgttgtcagaagtaagttggccgcagtgttatcactcatggttatggcagcactgcataattctcttactgtcatgccatccgtaagatgcttttctgtgactggtgagtactcaaccaagtcattctgagaatagtgtatgcggcgaccgagttgctcttgcccggcgtcaatacgggataataccgcgccacatagcagaactttaaaagtgctcatcattggaaaacgttcttcggggcgaaaactctcaaggatcttaccgctgttgagatccagttcgatgtaacccactcgtgcacccaactgatcttcagcatcttttactttcaccagcgtttctgggtgagcaaaaacaggaaggcaaaatgccgcaaaaaagggaataagggcgacacggaaatgttgaatactcatactcttcctttttcaatattattgaagcatttatcagggttattgtctcatgagcggatacatatttgaatgtatttagaaaaataaacaaataggggttccgcgcacatttccccgaaaagtgccacctgacgtctaagaaaccattattatcatgacattaacctataaaaataggcgtatcacgaggccctttcgtctcgcgcgtttcggtgatgacggtgaaaacctctgacacatgcagctcccggagacggtcacagcttgtctgtaagcggatgccgggagcagacaagcccgtcagggcgcgtcagcgggtgttggcgggtgtcggggctggcttaactatgcggcatcagagcagattgtactgagagtgcaccatatgcggtgtgaaataccgcacagatgcgtaaggagaaaataccgcatcaggcgccattcgccattcaggctgcgcaactgttgggaagggcgatcggtgcgggcctcttcgctattacgccagctggcgaaagggggatgtgctgcaaggcgattaagttgggtaacgccagggttttcccagtcacgacgttgtaaaacgacggcgcaaggaatggtgcatgcaaggagatggcgcccaacagtcccccggccacggggcctgccaccatacccacgccgaaacaagcgctcatgagcccgaagtggcgagcccgatcttccccatcggtgatgtcggcgatataggcgccagcaaccgcacctgtggcgccggtgatgccggccacgatgcgtccggcgtagaggcgattagtccaatttgttaaagacaggatatcagtggtccaggctctagttttgactcaacaatatcaccagctgaagcctatagagtacgagccatagataaaataaaagattttatttagtctccagaaaaaggggggaatgaaagaccccacctgtaggtttggcaagctagcttaagtaacgccattttgcaaggcatggaaaatacataactgagaatagagaagttcagatcaaggttaggaacagagagacagcagaatatgggccaaacaggatatctgtggtaagcagttcctgccccggctcagggccaagaacagatggtccccagatgcggtcccgccctcagcagtttctagagaaccatcagatgtttccagggtgccccaaggacctgaaatgaccctgtgccttatttgaactaaccaatcagttcgcttctcgcttctgttcgcgcgcttctgctccccgagctcaataaaagagcccacaacccctcactcggcgcgccagtcctccgatagactgcgtcgcccgggtacccgtattcccaataaagcctcttgctgtttgcatccgaatcgtggactcgctgatccttgggagggtctcctcagattgattgactgcccacctcgggggtctttcatttggaggttccaccgagatttggagacccctgcccagggaccaccgacccccccgccgggaggtaagctggccagcggtcgtttcgtgtctgtctctgtctttgtgcgtgtttgtgccggcatctaatgtttgcgcctgcgtctgtactagttagctaactagctctgtatctggcggacccgtggtggaactgacgagttcggaacacccggccgcaaccctgggagacgtcccagggacttcgggggccgtttttgtggcccgacctgagtcctaaaatcccgatcgtttaggactctttggtgcaccccccttagaggagggatatgtggttctggtaggagacgagaacctaaaacagttcccgcctccgtctgaatttttgctttcggtttgggaccgaagccgcgccgcgcgtcttgtctgctgcagcatcgttctgtgttgtctctgtctgactgtgtttctgtatttgtctgaaaatatgggcccgggctagcctgttaccactcccttaagtttgaccttaggtcactggaaagatgtcgagcggatcgctcacaaccagtcggtagatgtcaagaagagacgttgggttaccttctgctctgcagaatggccaacctttaacgtcggatggccgcgagacggcacctttaaccgagacctcatcacccaggttaagatcaaggtcttttcacctggcccgcatggacacccagaccaggtcccctacatcgtgacctgggaagccttggcttttgacccccctccctgggtcaagccctttgtacaccctaagcctccgcctcctcttcctccatccgccccgtctctcccccttgaacctcctcgttcgaccccgcctcgatcctccctttatccagccctcactccttctctaggcgcccccatatggccatatgagatcttatatggggcacccccgccccttgtaaacttccctgaccctgacatgacaagagttactaacagcccctctctccaagctcacttacaggctctctacttagtccagcacgaagtctggagacctctggcggcagcctaccaagaacaactggaccgaccggtggtacctcacccttaccgagtcggcgacacagtgtgggtccgccgacaccagactaagaacctagaacctcgctggaaaggaccttacacagtcctgctgaccacccccaccgccctcaaagtagacggcatcgcagcttggatacacgccgcccacgtgaaggctgccgaccccgggggtggaccatcctctagaccg

SEQ ID NO: 31 - DNA, 15 bp, Artificial Sequence
  Synthetic
agcatatttaacacc

SEQ ID NO: 32 - DNA, 21 bp, Artificial Sequence
  Synthetic
ttatataaggctggtgaattg

SEQ ID NO: 33 - DNA, 39 bp, Artificial Sequence
  Synthetic
gctgggcacccttcctcaaattccgggtatgcactcaac

SEQ ID NO: 34 - DNA, 15 bp, Artificial Sequence
  Synthetic
tcgggtcatgtatcc

SEQ ID NO: 35 - DNA, 18 bp, Artificial Sequence
  Synthetic
ttcaattatgaagcccaa

SEQ ID NO: 36 - DNA, 42 bp, Artificial Sequence
  Synthetic
gccagcagctcccagacaggggcccgcacagatacgcagtat

SEQ ID NO: 37 - protein, 27 aa, Artificial Sequence
  Synthetic
RAKRSGSGATNFSLLKQAGDVEENPGP

SEQ ID NO: 38 - DNA, 393 bp, Artificial Sequence
  Synthetic
atggcccttgaacatctgttgataatactgtggatgcaacttacctgggtatctggtcagcaattgaaccagtctccacagtccatgtttatccaagaaggggaggacgtgtccatgaattgtacaagctccagtatcttcaacacgtggctgtggtacaaacaggatcctggggaaggaccagtactgttgatagccctctataaggcgggcgaactgacatccaatggaagactcacagcccaattcggaattacccggaaggattctttcctcaacatctccgcgagtattccatctgatgtaggaatatacttctgtgcagggcatccgtctagcaacagtggatatgccctcaattttggaaagggcacctccctgctggttacccca

SEQ ID NO: 39 - DNA, 405 bp, Artificial Sequence
  Synthetic
atgggcacaagtttgctgtgctgggttgtgttgggctttctgggtacagatcatactggggcgggagtctctcaaagcccccgatacaaagtcactaaaagagggcaggatgtcgcgcttcgctgtgatcccattagcgggcatgtctccctttattggtaccggcaggctttgggacaaggaccggagttcctcacttacttcaactacgaagcgcagcaggacaagtccggtctgcctaatgatagattcagcgccgagagaccggagggcagtatctctactcttacgatacaaagaacggagcagcgagactctgctatgtatagatgtgcaagttctagccagacgggtgctcgcacggacactcaatatttcggtcctggtacaagattgaccgtcttg